European Patent Application EP 4 617 361 A1, published September 17, 2025. Title: 4-Hydroxybenzoic acid-producing Hydrogenophilus bacterium transformant. Applicant: UTILIZATION OF CARBON DIOXIDE INSTITUTE CO.,LTD. Application EP 22 965 101.3, filed November 8, 2022. The sequence listing filed with the application follows.

SEQUENCE LISTING (51 sequences)

SEQ ID NO: 1 - DNA, 579 bp, Shewanella algae
  source 1..579: mol_type = genomic DNA
atgagtgtgaccagtttaagctttccttatggtgaatcaattcagtggttttcgccagagcaatcacagcaacttcccgcagcgccattgcacgattggctgctggcgaccggcagtctcaccaagagactcaagagttgctgcaaccactttgaggtcaaactgctcggcgaagccatgctgccctcatccactcgggagtggcagggtaaggaacataaagccatctggatcagggaagtattgctctgcctggacggtactccctgggtctttggccgcaccctgatcccggcaaagctgctggagcaacagcagagactgggcaagttgggcacccgccccctgggagagttgttgttcggcgatatcggctttgaacccggcgccatagaggtcgccagtttcgacagccaatccaggattgcctccctcgccgactcactgtcacaacccaccactgaggcaatatggggcagaagacgttattttcacttccatgagcaacagctgattgtcggtgaaattttcctgccggcggcggttgccgccattaaccaagggccactaaccccctaa

SEQ ID NO: 2 - DNA, 510 bp, Cronobacter sakazakii
  source 1..510: mol_type = genomic DNA
atgtcccatcccgcgctgagacaactgcgcgcgttgtccttttttgacgatatcagcacgcttgatagttcgctgctcgactggctgatgctggaagattccatgacccgccgtttcgaaggcttttgcgagcgcgtgacggtcgacatgctgtttgagggctttgtcggccccgaggcgctggaggaagagggcgagtttttgcctgatgagccgcgctactggctgcgcgaaatcctgctgtgcggcgacggcgtgccgtggctggttgggcgcacgctggtgccggagtctacactttgtgggccggagctggcgttgcagcagctcggtaccacgccgctgggccgttatctgtttacctcatccaccctcacgcgtgattttatccagccgggccgcagcgacgaactctggggacgccgctctctgctgaggctttccggcaaaccgctgctgctgactgaactgtttttacctgcatcacccttgtacggagaggaaaaataa

SEQ ID NO: 3 - protein, 192 aa, Shewanella algae
MSVTSLSFPYGESIQWFSPEQSQQLPAAPLHDWLLATGSLTKRLKSCCNHFEVKLLGEAMLPSSTREWQGKEHKAIWIREVLLCLDGTPWVFGRTLIPAKLLEQQQRLGKLGTRPLGELLFGDIGFEPGAIEVASFDSQSRIASLADSLSQPTTEAIWGRRRYFHFHEQQLIVGEIFLPAAVAAINQGPLTP

SEQ ID NO: 4 - protein, 169 aa, Cronobacter sakazakii
MSHPALRQLRALSFFDDISTLDSSLLDWLMLEDSMTRRFEGFCERVTVDMLFEGFVGPEALEEEGEFLPDEPRYWLREILLCGDGVPWLVGRTLVPESTLCGPELALQQLGTTPLGRYLFTSSTLTRDFIQPGRSDELWGRRSLLRLSGKPLLLTELFLPASPLYGEEK

SEQ ID NO: 5 - DNA, 35 bp, synthetic construct
  source 1..35: mol_type = other DNA
ttttataacccgggccatcgactgcacggtgcacc

SEQ ID NO: 6 - DNA, 35 bp, synthetic construct
  source 1..35: mol_type = other DNA
tgctagcactgtttcctgtgtgaaattgttatccg

SEQ ID NO: 7 - DNA, 38 bp, synthetic construct
  source 1..38: mol_type = other DNA
ggaaacagtgctagcagatctggaggagaaaggcatat

SEQ ID NO: 8 - DNA, 72 bp, synthetic construct
  source 1..72: mol_type = other DNA
cagtgcggccgcaagcttgtcgacggagctcgaattcggatccgatatcagcatatgcgtttctcctccaga

SEQ ID NO: 9 - DNA, 80 bp, synthetic construct
  source 1..80: mol_type = other DNA
acaagcttgcggccgcactgcagcaccatcaccaccatcattgataagatccggctgctaacaaagcccgaaaggaagct

SEQ ID NO: 10 - DNA, 63 bp, synthetic construct
  source 1..63: mol_type = other DNA
tatttgaatcgagttattgctcagcggtggcagcagccaactcagcttcctttcgggctttgt

SEQ ID NO: 11 - DNA, 35 bp, synthetic construct
  source 1..35: mol_type = other DNA
taactcgattcaaataaaacgaaaggctcagtcga

SEQ ID NO: 12 - DNA, 35 bp, synthetic construct
  source 1..35: mol_type = other DNA
cctagatccgcggagtttgtagaaacgcaaaaagg

SEQ ID NO: 13 - DNA, 35 bp, synthetic construct
  source 1..35: mol_type = other DNA
acaaactccgcggatctaggtgaagatcctttttg

SEQ ID NO: 14 - DNA, 35 bp, synthetic construct
  source 1..35: mol_type = other DNA
cgtccgcggccagcaaaaggccaggaaccgtaaaa

SEQ ID NO: 15 - DNA, 35 bp, synthetic construct
  source 1..35: mol_type = other DNA
ttgctggccgcggacgtagaaagcctgtccgcaga

SEQ ID NO: 16 - DNA, 35 bp, synthetic construct
  source 1..35: mol_type = other DNA
ggcccgggttataaaagccagtcattaggcctatc

SEQ ID NO: 17 - DNA, 35 bp, synthetic construct
  source 1..35: mol_type = other DNA
aattgtcagataggcctaatgactggcttttataa

SEQ ID NO: 18 - DNA, 35 bp, synthetic construct
  source 1..35: mol_type = other DNA
tgacgccagaagcattggtgcaccgtgcagtcgat

SEQ ID NO: 19 - DNA, 19 bp, synthetic construct
  source 1..19: mol_type = other DNA
gatctggaggagaaacgca

SEQ ID NO: 20 - DNA, 17 bp, synthetic construct
  source 1..17: mol_type = other DNA
tatgcgtttctcctcca

SEQ ID NO: 21 - DNA, 35 bp, synthetic construct
  source 1..35: mol_type = other DNA
gaggccatctaggccatgagtaagtctgacggaac

SEQ ID NO: 22 - DNA, 35 bp, synthetic construct
  source 1..35: mol_type = other DNA
atccggcacccatatctgaaccggacgcaaacccg

SEQ ID NO: 23 - DNA, 35 bp, synthetic construct
  source 1..35: mol_type = other DNA
ttcagatatgggtgccggatacccgccgcccgggc

SEQ ID NO: 24 - DNA, 35 bp, synthetic construct
  source 1..35: mol_type = other DNA
aaggccttcatggccttatttcgcgattcccaaga

SEQ ID NO: 25 - DNA, 549 bp, Aquitalea magnusonii
  source 1..549: mol_type = genomic DNA
atgtccggctttggcataatgcgcgccatgattcaggatacacactggctgccgcagccccccgaccttgcccccggcctgctggccttcgtcagcgaagccggctcgctgaccgagcggctgctggccaccggccaccgcttcggcgtgcaggtattgtcacaaggcgcaagcccggccaacccggacgagcccgccctgcttgccctgccagccgacagcctgctgtatgcccgccatgtgctgctgaccctggatgacaccccggtggtgtacgcgcgcagcattgcccggctggactgcccggtgtggcagcccattctggaccgtggcagccgctcgctcggactcaccctgtttggcggcctgccgcagctgcagcgcggcccgctgcactatcagcaactggggccggcccatcccctgcatcaggcctgtgcaagcgatagcaccagcctgacggcacggcgctgccgctttgtgctggatgaagccccgatggtggtgtgcgaggtgttcctgcccgccctgaaagattttgcccgatga

SEQ ID NO: 26 - DNA, 663 bp, Cupriavidus necator
  source 1..663: mol_type = genomic DNA
atgagcgcgcagtccgcgcgccgctgcagctggagcccgcacctggcctttgatgcagccatcacgcccaacctgcggcgctgggtgaccggtgacgacggctcgctgaccgcgcgcctggtggcagcatcggagcgctttcgcgtggcgcgcctgctgcagcgcccgcagcgcccgctcgccgatgaatggcaggtgctgggccagcacgaccgcacccccgcgctgacgcgcgaggtgctgctgatctgcgacgatattcccgccatatttgcccatactgtggtgcgccagcgccatgcgcgccgcgactggccgttcctgcgcgggctgggcgagcgcccgctgggcggccggctgtttgtcgacccggcggtggcgcgcgagccgttccagtttgcgcggctgctgccgcaccatccgctgcgccaggccttgcagcgtgtgctgccggccatggcgccactgcccatgctgccggcgcggcgctcggtgttccggcgcggcgacggcgtcatgctcgtgacagaagtgttcctgccggacctgctgtcgcggccatccccggggaccgaggcgattccgtatcccaggtatttgcggactacagaccgaagcccctctacacacactaccgaaaccaagaaagagaccacgagatga

SEQ ID NO: 27 - DNA, 528 bp, Mixta theicola
  source 1..528: mol_type = genomic DNA
atgtccgataacgcgctttccctgctgcgcgccattgcctggcttcccacctcgtcacctgcgctgtccgctcctttgctcgactggctattggaagaggattcgatgacaaagcgttttgagcgccactgtcagaaagttaccgtagagccgcagtttgaaggcttcgttagcgctgacgctatcgctgaggaactgccgtttctgccgctggagccgcgctactggctgcgcgagatcattttgtcgggtgatggcgttccctggctggctggccgcacggtggtgccggcatcgacgctggacgggccggaaatgatgctcagccagctgggcacccgtccgctgggccggtatctcttttcttcctccacgctaacgcgtgactttatcgatcctggggtcgctgccgcgctgtggggacgccgctcgcgcctgcgtttatcgggcaaaccgctgctattaaccgaactgtttttacccgctgcgccgctttatcaaagcctgcctggagagccaagtgagtaa

SEQ ID NO: 28 - DNA, 510 bp, Proteus mirabilis
  source 1..510: mol_type = genomic DNA
atgtttaaaaaatccataattactcacgcacctattcactggttatcagatgaagagcgtgaagaagtcgcagaaaataccttaagttggctgctggaattaggttcaatgacacgacgttttgagcaacattgccatcaagtgacggtaatgccatatcaagaaggttttattgaatatatcgagcctgctgatgaacaaaagtgtttaccttatagccgacgctattggctaagagaaatcgtcctttgtggggataatgtaccttggttattagggcgaacattagtgccggaagagacattaacgggtgaagatcgccaattagtgaatttgcgtacggtgccattaggacgttatctgttccaggaaacaaccttaagtcgtgattttattcatattgggcaacaaaatggacattggttacgtcgttcccgtttccagctttcagataaacctttattattaactgaggtgtttttgcctgcatcacctgtatataagcagtag

SEQ ID NO: 29 - DNA, 564 bp, Pseudomonas fluorescens
  source 1..564: mol_type = genomic DNA
atgccgcactcaatcgcccttcccgatgcttgccaatggctgacccagagccttctgagccctttgcccgcgcctttgaccctcgattggctgttcgacgaaggctcactgacgcgccggctcacgcggctgtccaacgatgagttcagcgtcacgccgctgttcgaaggctggcagccgttgcgcgaggatgaatgtgcggcgctgggcctggccccggccactgtcggttgggtgcgcgaggtgtatctgcgcgggcatgcccagccgtgggtgttcgcccgcagcgtggcggcgcgcagtgccctgcagggcgacgggttgcatatggacgcgttgggcagccgttcgttgggcgagttgctgttttgcgatcacgccttcacccgccagcccatcgaggtgtgccattacccacggcaatggctgccgagcgcggaccaggccgacggcttgtgggggcgccgctcacgctttgatcgcgggccgctgagtgtgctggtggcggaaattttcctgccgagcttctggcacgcgttgcatgaccatccggagaactgctga

SEQ ID NO: 30 - DNA, 552 bp, Azotobacter vinelandii
  source 1..552: mol_type = genomic DNA
atgaccgctgctcccgctttccaatggctcggcgccgaccaactgcatcccgcccccccggccgtcctggccgactggctgttcgacagcggctcgctgacccgccggctgaccgccctttccgccggccgtttcgccgtgacgccgctggccgaaggctggcaggtgctgcgcgacgacgaatgcgccgccctcgacgtggtgccgggcagcaccggctgggtacgcgaggtctacctgctcggcgccgagcggccctgggtgttcgcccgcagcgtggcggcccgcgaggctctggcgggtttctccggcgtactcgccgaactcggccggcggcccctcggcgaactgctgttcagcgacccggccttcgcccgcggcccgctgcaggccacgcactatccgccggactggctgccggccgggatacgctgccccggactctggggacggcgctcccgtttccaccgggaaaccctgagcgtgctggtggcggaagtcttcctgccggagctctggcgctaccagggaatcgacccggacaccctataa

SEQ ID NO: 31 - DNA, 618 bp, Hydrogenophilus thermoluteolus
  source 1..618: mol_type = genomic DNA
atgcgtgaggcatccgctgctggcttccctgcacactggtatgggaatgcagttgccgttcttcctgcgtggcgccgttggctctttggcagcggctcccttaccgcccgtctcgaagcacgttgccagcagttgcttcgtgtggcgccaatcgcgcaagggcgtgcgcccgttgccgccgacgagcggtcgctcttgggcgtctcaacgcgcatcgcctgggtgcgcgaagtcgcgctcatcgcagacgatgttgcggtggtctttgcccggtccgtgctcgtaccctcggcgcgcgccgcctggccgctctttttccgtgtcgggactcggccgcttggggcactgctcttcgaagattctgcggtatttcgcggtccgatcgaagcggcgcgcatcgattcacgacataccttgtggcgccgcgccgcgcaccatgcgctgttgcgctcgggtgaggagcgcgccgcgctctgggcgcgccgttcgtgcttttggcggtttggtaagcccttgctggtccaagaactctttttgcccggtatcgcgacactcgatccggggttgcgccaagcgggtgcgtggccgtcgcatcgcgctgtgaacccggtagaatga

SEQ ID NO: 32 - DNA, 44 bp, synthetic construct
  source 1..44: mol_type = other DNA
gcagatctggaggagaaacgcatatgagtgtgaccagtttaagc

SEQ ID NO: 33 - DNA, 43 bp, synthetic construct
  source 1..43: mol_type = other DNA
cttgtcgacggagctcgaattctcaaggcgtaagttggccttg

SEQ ID NO: 34 - DNA, 44 bp, synthetic construct
  source 1..44: mol_type = other DNA
cagatctggaggagaaacgcatatgtcccatcccgcgctgagac

SEQ ID NO: 35 - DNA, 42 bp, synthetic construct
  source 1..42: mol_type = other DNA
gcttgtcgacggagctcgaattcttatttttcctctccgtac

SEQ ID NO: 36 - DNA, 44 bp, synthetic construct
  source 1..44: mol_type = other DNA
cagatctggaggagaaacgcatatgtccggctttggcataatgc

SEQ ID NO: 37 - DNA, 43 bp, synthetic construct
  source 1..43: mol_type = other DNA
cttgtcgacggagctcgaattctcatcgggcaaaatctttcag

SEQ ID NO: 38 - DNA, 41 bp, synthetic construct
  source 1..41: mol_type = other DNA
gatctggaggagaaacgcatatgagcgcgcagtccgcgcgc

SEQ ID NO: 39 - DNA, 41 bp, synthetic construct
  source 1..41: mol_type = other DNA
gtcgacggagctcgaattctcatctcgtggtctctttcttg

SEQ ID NO: 40 - DNA, 44 bp, synthetic construct
  source 1..44: mol_type = other DNA
gatctggaggagaaacgcatatgtccgataacgcgctttccctg

SEQ ID NO: 41 - DNA, 43 bp, synthetic construct
  source 1..43: mol_type = other DNA
gtcgacggagctcgaattcttactcacttggctctccaggcag

SEQ ID NO: 42 - DNA, 43 bp, synthetic construct
  source 1..43: mol_type = other DNA
gatctggaggagaaacgcatatgtttaaaaaatccataattac

SEQ ID NO: 43 - DNA, 43 bp, synthetic construct
  source 1..43: mol_type = other DNA
gcttgtcgacggagctcgaattcctactgcttatatacaggtg

SEQ ID NO: 44 - DNA, 44 bp, synthetic construct
  source 1..44: mol_type = other DNA
cagatctggaggagaaacgcatatgccgcactcaatcgcccttc

SEQ ID NO: 45 - DNA, 44 bp, synthetic construct
  source 1..44: mol_type = other DNA
gcttgtcgacggagctcgaattctcagcagttctccggatggtc

SEQ ID NO: 46 - DNA, 43 bp, synthetic construct
  source 1..43: mol_type = other DNA
cagatctggaggagaaacgcatatgaccgctgctcccgctttc

SEQ ID NO: 47 - DNA, 41 bp, synthetic construct
  source 1..41: mol_type = other DNA
cttgtcgacggagctcgaattcttatagggtgtccgggtcg

SEQ ID NO: 48 - DNA, 44 bp, synthetic construct
  source 1..44: mol_type = other DNA
cagatctggaggagaaacgcatatgcgtgaggcatccgctgctg

SEQ ID NO: 49 - DNA, 44 bp, synthetic construct
  source 1..44: mol_type = other DNA
cttgtcgacggagctcgaattctcattctaccgggttcacagcg

SEQ ID NO: 50 - DNA, 20 bp, synthetic construct
  source 1..20: mol_type = other DNA
gaattcgagctccgtcgaca

SEQ ID NO: 51 - DNA, 20 bp, synthetic construct
  source 1..20: mol_type = other DNA
atgcgtttctcctccagatc